European Patent Application EP 4 353 244 A1, published April 17, 2024. Title: THE COMPOSITION FOR PREVENTING OR TREATING VASCULAR DEMENTIA. Applicant: SEOUL NATIONAL UNIVERSITY R&DB FOUNDATION. The sequence listing filed with the application follows.

SEQUENCE LISTING (24 sequences)

SEQ ID NO: 1 - DNA, 20 bp, synthetic construct
  source 1..20: mol_type = other DNA
gtcagtggtggacctgacct

SEQ ID NO: 2 - DNA, 20 bp, synthetic construct
  source 1..20: mol_type = other DNA
caccaccctgttgctgtagc

SEQ ID NO: 3 - DNA, 20 bp, synthetic construct
  source 1..20: mol_type = other DNA
caacctgcagattcgagaaa

SEQ ID NO: 4 - DNA, 20 bp, synthetic construct
  source 1..20: mol_type = other DNA
gtcctgcctcacatcacatc

SEQ ID NO: 5 - DNA, 21 bp, synthetic construct
  source 1..21: mol_type = other DNA
cacctgtgccagcctttctta

SEQ ID NO: 6 - DNA, 20 bp, synthetic construct
  source 1..20: mol_type = other DNA
tttcctcccaccctgtgtct

SEQ ID NO: 7 - DNA, 20 bp, synthetic construct
  source 1..20: mol_type = other DNA
agtctccaagcgacgaaaaa

SEQ ID NO: 8 - DNA, 20 bp, synthetic construct
  source 1..20: mol_type = other DNA
gcaagaagcctctccttgaa

SEQ ID NO: 9 - DNA, 21 bp, synthetic construct
  source 1..21: mol_type = other DNA
aggtattacgagactggctcc

SEQ ID NO: 10 - DNA, 22 bp, synthetic construct
  source 1..22: mol_type = other DNA
tcccgcttatactgggctattt

SEQ ID NO: 11 - DNA, 21 bp, synthetic construct
  source 1..21: mol_type = other DNA
agaactttgccgttgaagctg

SEQ ID NO: 12 - DNA, 23 bp, synthetic construct
  source 1..23: mol_type = other DNA
ccagagggagtgaatccagatta

SEQ ID NO: 13 - DNA, 19 bp, synthetic construct
  source 1..19: mol_type = other DNA
cggaccagtacccgcacct

SEQ ID NO: 14 - DNA, 21 bp, synthetic construct
  source 1..21: mol_type = other DNA
ggcgcttgtcactttcgttca

SEQ ID NO: 15 - DNA, 20 bp, synthetic construct
  source 1..20: mol_type = other DNA
ggagacggcgaatgtgactt

SEQ ID NO: 16 - DNA, 23 bp, synthetic construct
  source 1..23: mol_type = other DNA
gaactcgtggcaggcagtagtaa

SEQ ID NO: 17 - DNA, 22 bp, synthetic construct
  source 1..22: mol_type = other DNA
tacacttgctattacaaccaca

SEQ ID NO: 18 - DNA, 20 bp, synthetic construct
  source 1..20: mol_type = other DNA
atcctccacgatgactaaat

SEQ ID NO: 19 - DNA, 22 bp, synthetic construct
  source 1..22: mol_type = other DNA
ggttgctgcaagcactcatcac

SEQ ID NO: 20 - DNA, 22 bp, synthetic construct
  source 1..22: mol_type = other DNA
cacgccattgttctcttccagg

SEQ ID NO: 21 - DNA, 22 bp, synthetic construct
  source 1..22: mol_type = other DNA
tgccaacagaggacatcagcct

SEQ ID NO: 22 - DNA, 22 bp, synthetic construct
  source 1..22: mol_type = other DNA
cagctcagacttggagaggtga

SEQ ID NO: 23 - DNA, 21 bp, synthetic construct
  source 1..21: mol_type = other DNA
cagaatgcactgttacctgga

SEQ ID NO: 24 - DNA, 21 bp, synthetic construct
  source 1..21: mol_type = other DNA
gctgatcccaattctctttca